European Patent Application EP 4 778 941 A1, published July 22, 2026. Title: HER3/MET结合分子及其医药用途. Applicant: 江苏恒瑞医药股份有限公司. Application WO. The sequence listing filed with the application follows.

SEQUENCE LISTING (98 sequences)

SEQ ID NO: 1 - protein, 117 aa, synthetic construct
  source 1..117: note = A13 VH
QVQLVQSGAEVKKPGASVKVSCEASGYTFTSYGFSWVRQAPGQGLEWMGWISASNGNTYYAQKLQGRVTMTTDTSTSSAYMELRSLRSDDTAVYYCARVYADYADYWGQGTLVTVSS

SEQ ID NO: 2 - protein, 107 aa, synthetic construct
  source 1..107: note = A13 VL
DIQMTQSPSSVSASVGDRVTITCRASQGINTWLAWYQQKPGKAPKLLIYAASSLKSGVPSRFSGSGSGADFTLTISSLQPEDFATYYCQQANSFPLTFGGGTKVEIK

SEQ ID NO: 3 - protein, 120 aa, synthetic construct
  source 1..120: note = S3 VH
QVQLVESGGGVVQPGRSLRLSCAASGFSLSNYGVHWVRQAPGKGLEWLAVIWSGGSTNYAAAFVSRLTISKDNSKNTVYLQMNSLRAEDTAVYYCARNHDNPYNYAMDYWGQGTTVTVSS

SEQ ID NO: 4 - protein, 111 aa, synthetic construct
  source 1..111: note = S3 VL
DIVLTQSPDSLAVSLGERATINCRADKSVSTSTYNYLHWYQQKPGQPPKLLIYLASNLASGVPDRFSGSGSGTDFTLTISSLQAEDVAVYYCQHSRDLPPTFGQGTKLEIK

SEQ ID NO: 5 - protein, 135 aa, synthetic construct
  source 1..135: note = A9 VH
QVQLQESGPGLVKPSQTLSLTCTVSGGSISSGGYYWSWIRQHPGKGLEWIGYIYYSGSTYYNPSLKSRVTISVDTSKNQFSLKLSSVTAADTAVYYCARDGPLGYCSSTSCPVTGEYYYYGMDVWGQGTTVTVSS

SEQ ID NO: 6 - protein, 109 aa, synthetic construct
  source 1..109: note = A9 VL
EIVLTQSPGTLSLSPGERATLSCRASQSVSNNYLAWYQQKPGQAPRLLIFGASSRATGIPDRFSGSGSGTDFTLTISRLEPEDFAVYYCQQYDISPMYSFGQGTKLEMK

SEQ ID NO: 7 - protein, 121 aa, synthetic construct
  source 1..121: note = P8 VH
EVQLLESGGGLVQPGGSLRLSCAASGFTFSSYAMSWVRQAPGKGLEWVSAISGSGGSTYYADSVKGRFTISRDNSKNTLYLQMNSLRAEDTAVYYCAKDHYYDSSGYLDYWGQGTLVTVSS

SEQ ID NO: 8 - protein, 111 aa, synthetic construct
  source 1..111: note = P8 VL
NFMLTQPHSVSESPGKTVTISCTRSSGSIAFDYVQWYQQRPGSAPTTVIYEDNQRPSGVPDRFSASIDSSSNSASLTISALKTEDEADYYCQSYDNSNSWVFGGGTKLTVL

SEQ ID NO: 9 - protein, 119 aa, synthetic construct
  source 1..119: note = P3 VH
QVQLQESGPGLVKPSATLSLTCAVSGGSISSNHWWSWVRQSPGKGLEWIGEIYTYGGANYNPSLKSRVDISMDKSKNQFSLHLSSVTAADTAVYYCGRHLTGYDCFDIWGQGTLVTVSS

SEQ ID NO: 10 - protein, 110 aa, synthetic construct
  source 1..110: note = P3 VL
QAVLTQPSSVSGAPGQRVTISCTGSSSNIGAGYDVHWYQQLPGTAPKLLIYGNSNRPSGVPDRFSGSKSGTSASLAITGLQAEDEADYYCQSYDSSLSGVFGTGTQLTVL

SEQ ID NO: 11 - protein, 119 aa, synthetic construct [sequence omitted]

SEQ ID NO: 12 - protein, 113 aa, synthetic construct [sequence omitted]

SEQ ID NO: 13 - protein, 117 aa, synthetic construct
  source 1..117: note = A VH
QVQLVQSGGGLVQPGRSLRLSCAASGFTFDDYAMHWVRQAPGKGLEWVSGISWNSGSIGYADSVKGRFTISRDNAKNSLYLQMNSLRAEDTALYYCAKEGLPGLDYWGQGTLVTVSS

SEQ ID NO: 14 - protein, 108 aa, synthetic construct
  source 1..108: note = A VL
DIQMTQSPSSLSASIGDRATITCRASQHVGTYLNWYQQKPGKTPKLLISGAANLQSGVPSRFSGSGSGTDFTLTISSLQPEDFATYYCQQSYNTPPFSFGQGTKVEIK

SEQ ID NO: 15 - protein, 5 aa, synthetic construct
  source 1..5: note = CDR
SYGFS

SEQ ID NO: 16 - protein, 17 aa, synthetic construct
  source 1..17: note = CDR
WISASNGNTYYAQKLQG

SEQ ID NO: 17 - protein, 8 aa, synthetic construct
  source 1..8: note = CDR
VYADYADY

SEQ ID NO: 18 - protein, 11 aa, synthetic construct
  source 1..11: note = CDR
RASQGINTWLA

SEQ ID NO: 19 - protein, 7 aa, synthetic construct
  source 1..7: note = CDR
AASSLKS

SEQ ID NO: 20 - protein, 9 aa, synthetic construct
  source 1..9: note = CDR
QQANSFPLT

SEQ ID NO: 21 - protein, 5 aa, synthetic construct
  source 1..5: note = CDR
NYGVH

SEQ ID NO: 22 - protein, 16 aa, synthetic construct
  source 1..16: note = CDR
VIWSGGSTNYAAAFVS

SEQ ID NO: 23 - protein, 12 aa, synthetic construct
  source 1..12: note = CDR
NHDNPYNYAMDY

SEQ ID NO: 24 - protein, 15 aa, synthetic construct
  source 1..15: note = CDR
RADKSVSTSTYNYLH

SEQ ID NO: 25 - protein, 7 aa, synthetic construct
  source 1..7: note = CDR
LASNLAS

SEQ ID NO: 26 - protein, 9 aa, synthetic construct
  source 1..9: note = CDR
QHSRDLPPT

SEQ ID NO: 27 - protein, 7 aa, synthetic construct
  source 1..7: note = CDR
SGGYYWS

SEQ ID NO: 28 - protein, 16 aa, synthetic construct
  source 1..16: note = CDR
YIYYSGSTYYNPSLKS

SEQ ID NO: 29 - protein, 25 aa, synthetic construct
  source 1..25: note = CDR
DGPLGYCSSTSCPVTGEYYYYGMDV

SEQ ID NO: 30 - protein, 12 aa, synthetic construct
  source 1..12: note = CDR
RASQSVSNNYLA

SEQ ID NO: 31 - protein, 7 aa, synthetic construct
  source 1..7: note = CDR
GASSRAT

SEQ ID NO: 32 - protein, 10 aa, synthetic construct
  source 1..10: note = CDR
QQYDISPMYS

SEQ ID NO: 33 - protein, 5 aa, synthetic construct
  source 1..5: note = CDR
SYAMS

SEQ ID NO: 34 - protein, 17 aa, synthetic construct
  source 1..17: note = CDR
AISGSGGSTYYADSVKG

SEQ ID NO: 35 - protein, 12 aa, synthetic construct
  source 1..12: note = CDR
DHYYDSSGYLDY

SEQ ID NO: 36 - protein, 13 aa, synthetic construct
  source 1..13: note = CDR
TRSSGSIAFDYVQ

SEQ ID NO: 37 - protein, 7 aa, synthetic construct
  source 1..7: note = CDR
EDNQRPS

SEQ ID NO: 38 - protein, 10 aa, synthetic construct
  source 1..10: note = CDR
QSYDNSNSWV

SEQ ID NO: 39 - protein, 6 aa, synthetic construct
  source 1..6: note = CDR
SNHWWS

SEQ ID NO: 40 - protein, 16 aa, synthetic construct
  source 1..16: note = CDR
EIYTYGGANYNPSLKS

SEQ ID NO: 41 - protein, 10 aa, synthetic construct
  source 1..10: note = CDR
HLTGYDCFDI

SEQ ID NO: 42 - protein, 14 aa, synthetic construct
  source 1..14: note = CDR
TGSSSNIGAGYDVH

SEQ ID NO: 43 - protein, 7 aa, synthetic construct
  source 1..7: note = CDR
GNSNRPS

SEQ ID NO: 44 - protein, 10 aa, synthetic construct
  source 1..10: note = CDR
QSYDSSLSGV

SEQ ID NO: 45 - protein, 5 aa, synthetic construct
  source 1..5: note = CDR
SYWLH

SEQ ID NO: 46 - protein, 17 aa, synthetic construct
  source 1..17: note = CDR
MIDPSNSDTRFNPNFKD

SEQ ID NO: 47 - protein, 10 aa, synthetic construct
  source 1..10: note = CDR
YRSYVTPLDY

SEQ ID NO: 48 - protein, 17 aa, synthetic construct
  source 1..17: note = CDR
KSSQSLLYTSSQKNYLA

SEQ ID NO: 49 - protein, 7 aa, synthetic construct
  source 1..7: note = CDR
WASTRES

SEQ ID NO: 50 - protein, 9 aa, synthetic construct
  source 1..9: note = CDR
QQYYAYPWT

SEQ ID NO: 51 - protein, 5 aa, synthetic construct
  source 1..5: note = CDR
DYAMH

SEQ ID NO: 52 - protein, 17 aa, synthetic construct
  source 1..17: note = CDR
GISWNSGSIGYADSVKG

SEQ ID NO: 53 - protein, 8 aa, synthetic construct
  source 1..8: note = CDR
EGLPGLDY

SEQ ID NO: 54 - protein, 11 aa, synthetic construct
  source 1..11: note = CDR
RASQHVGTYLN

SEQ ID NO: 55 - protein, 7 aa, synthetic construct
  source 1..7: note = CDR
GAANLQS

SEQ ID NO: 56 - protein, 10 aa, synthetic construct
  source 1..10: note = CDR
QQSYNTPPFS

SEQ ID NO: 57 - protein, 446 aa, synthetic construct
  source 1..446: note = 2232-01 H1
QVQLVQSGAEVKKPGASVKVSCEASGYTFTSYGFSWVRQAPGQGLEWMGWISASNGNTYYAQKLQGRVTMTTDTSTSSAYMELRSLRSDDTAVYYCARVYADYADYWGQGTLVTVSSGGGGSSGAPRFLTRPKASVVSVGKDATLSCQIVGNPFPQVSWEKDKQPVTAGVRFRLAQDGDLYRLKILDLQLSDSGQYVCRARNAHGEAFACLGLQVDAEADKTHTCPPCPAPELLGGPSVFLFPPKPKDTLMISRTPEVTCVVVDVSHEDPEVKFNWYVDGVEVHNAKTKPREEQYNSTYRVVSVLTVLHQDWLNGKEYKCKVSNKALPAPIEKTISKAKGQPREPQVYTLPPCREEMTKNQVSLWCLVKGFYPSDIAVEWESNGQPENNYKTTPPVLDSDGSFFLYSKLTVDKSRWQQGNVFSCSVMHEALHNHYTQKSLSLSPGK

SEQ ID NO: 58 - protein, 210 aa, synthetic construct
  source 1..210: note = 2232-01 L1
DIQMTQSPSSVSASVGDRVTITCRASQGINTWLAWYQQKPGKAPKLLIYAASSLKSGVPSRFSGSGSGADFTLTISSLQPEDFATYYCQQANSFPLTFGGGTKVEIKGGGGSGIPPKIECLPIDISIDEGKVLTVASAFTGEPTPEVTWSTGGRKIHSQEQGRFHIENTDDSTTLTIKDVQKQDGGLYTLTLRNEFGSDSATVNIHIRSI

SEQ ID NO: 59 - protein, 447 aa, synthetic construct
  source 1..447: note = 2232-01 H2
QVQLVQSGGGLVQPGRSLRLSCAASGFTFDDYAMHWVRQAPGKGLEWVSGISWNSGSIGYADSVKGRFTISRDNAKNSLYLQMNSLRAEDTALYYCAKEGLPGLDYWGQGTLVTVSSASTKGPSVFPLAPSSKSTSGGTAALGCLVKDYFPEPVTVSWNSGALTSGVHTFPAVLQSSGLYSLSSVVTVPSSSLGTQTYICNVNHKPSNTKVDKKVEPKSCDKTHTCPPCPAPELLGGPSVFLFPPKPKDTLMISRTPEVTCVVVDVSHEDPEVKFNWYVDGVEVHNAKTKPREEQYNSTYRVVSVLTVLHQDWLNGKEYKCKVSNKALPAPIEKTISKAKGQPREPQVCTLPPSREEMTKNQVSLSCAVKGFYPSDIAVEWESNGQPENNYKTTPPVLDSDGSFFLVSKLTVDKSRWQQGNVFSCSVMHEALHNHYTQKSLSLSPGK

SEQ ID NO: 60 - protein, 215 aa, synthetic construct
  source 1..215: note = 2232-01 L2
DIQMTQSPSSLSASIGDRATITCRASQHVGTYLNWYQQKPGKTPKLLISGAANLQSGVPSRFSGSGSGTDFTLTISSLQPEDFATYYCQQSYNTPPFSFGQGTKVEIKRTVAAPSVFIFPPSDEQLKSGTASVVCLLNNFYPREAKVQWKVDNALQSGNSQESVTEQDSKDSTYSLSSTLTLSKADYEKHKVYACEVTHQGLSSPVTKSFNRGEC

SEQ ID NO: 61 - protein, 449 aa, synthetic construct
  source 1..449: note = 2232-02 H1
QVQLVESGGGVVQPGRSLRLSCAASGFSLSNYGVHWVRQAPGKGLEWLAVIWSGGSTNYAAAFVSRLTISKDNSKNTVYLQMNSLRAEDTAVYYCARNHDNPYNYAMDYWGQGTTVTVSSGGGGSSGAPRFLTRPKASVVSVGKDATLSCQIVGNPFPQVSWEKDKQPVTAGVRFRLAQDGDLYRLKILDLQLSDSGQYVCRARNAHGEAFACLGLQVDAEADKTHTCPPCPAPELLGGPSVFLFPPKPKDTLMISRTPEVTCVVVDVSHEDPEVKFNWYVDGVEVHNAKTKPREEQYNSTYRVVSVLTVLHQDWLNGKEYKCKVSNKALPAPIEKTISKAKGQPREPQVYTLPPCREEMTKNQVSLWCLVKGFYPSDIAVEWESNGQPENNYKTTPPVLDSDGSFFLYSKLTVDKSRWQQGNVFSCSVMHEALHNHYTQKSLSLSPGK

SEQ ID NO: 62 - protein, 214 aa, synthetic construct
  source 1..214: note = 2232-02 L1
DIVLTQSPDSLAVSLGERATINCRADKSVSTSTYNYLHWYQQKPGQPPKLLIYLASNLASGVPDRFSGSGSGTDFTLTISSLQAEDVAVYYCQHSRDLPPTFGQGTKLEIKGGGGSGIPPKIECLPIDISIDEGKVLTVASAFTGEPTPEVTWSTGGRKIHSQEQGRFHIENTDDSTTLTIKDVQKQDGGLYTLTLRNEFGSDSATVNIHIRSI

SEQ ID NO: 63 - protein, 97 aa, synthetic construct
  source 1..97: note = Obscurin-O
SGAPRFLTRPKASVVSVGKDATLSCQIVGNPFPQVSWEKDKQPVTAGVRFRLAQDGDLYRLKILDLQLSDSGQYVCRARNAHGEAFACLGLQVDAEA

SEQ ID NO: 64 - protein, 98 aa, synthetic construct
  source 1..98: note = Titin-T
GIPPKIECLPIDISIDEGKVLTVASAFTGEPTPEVTWSTGGRKIHSQEQGRFHIENTDDSTTLTIKDVQKQDGGLYTLTLRNEFGSDSATVNIHIRSI

SEQ ID NO: 65 - protein, 103 aa, synthetic construct
  source 1..103: note = CH1
ASTKGPSVFPLAPSSKSTSGGTAALGCLVKDYFPEPVTVSWNSGALTSGVHTFPAVLQSSGLYSLSSVVTVPSSSLGTQTYICNVNHKPSNTKVDKKVEPKSC

SEQ ID NO: 66 - protein, 107 aa, synthetic construct [sequence omitted]

SEQ ID NO: 67 - protein, 227 aa, synthetic construct
  source 1..227: note = IgG1 Fc1
DKTHTCPPCPAPELLGGPSVFLFPPKPKDTLMISRTPEVTCVVVDVSHEDPEVKFNWYVDGVEVHNAKTKPREEQYNSTYRVVSVLTVLHQDWLNGKEYKCKVSNKALPAPIEKTISKAKGQPREPQVYTLPPCREEMTKNQVSLWCLVKGFYPSDIAVEWESNGQPENNYKTTPPVLDSDGSFFLYSKLTVDKSRWQQGNVFSCSVMHEALHNHYTQKSLSLSPGK

SEQ ID NO: 68 - protein, 227 aa, synthetic construct
  source 1..227: note = IgG1 Fc2
DKTHTCPPCPAPELLGGPSVFLFPPKPKDTLMISRTPEVTCVVVDVSHEDPEVKFNWYVDGVEVHNAKTKPREEQYNSTYRVVSVLTVLHQDWLNGKEYKCKVSNKALPAPIEKTISKAKGQPREPQVCTLPPSREEMTKNQVSLSCAVKGFYPSDIAVEWESNGQPENNYKTTPPVLDSDGSFFLVSKLTVDKSRWQQGNVFSCSVMHEALHNHYTQKSLSLSPGK

SEQ ID NO: 69 - protein, 4 aa, synthetic construct
  source 1..4: note = linker
GGFG

SEQ ID NO: 70 - protein, 108 aa, synthetic construct
  source 1..108: note = A VL T94V
DIQMTQSPSSLSASIGDRATITCRASQHVGTYLNWYQQKPGKTPKLLISGAANLQSGVPSRFSGSGSGTDFTLTISSLQPEDFATYYCQQSYNVPPFSFGQGTKVEIK

SEQ ID NO: 71 - protein, 117 aa, synthetic construct
  source 1..117: note = A13 E23K/S78T/A69T/N30 VH
QVQLVQSGAEVKKPGASVKVSCKASGYTFTSYGFSWVRQAPGQGLEWMGWISASNGNTYYAQKLQGRVTMTTDTSTSTAYMELRSLRSDDTAVYYCARVYADYADYWGQGTLVTVSS

SEQ ID NO: 72 - protein, 107 aa, synthetic construct
  source 1..107: note = A13 E23K/S78T/A69T/N30 VL
DIQMTQSPSSVSASVGDRVTITCRASQGISTWLAWYQQKPGKAPKLLIYAASSLKSGVPSRFSGSGSGTDFTLTISSLQPEDFATYYCQQANSFPLTFGGGTKVEIK

SEQ ID NO: 73 - protein, 10 aa, synthetic construct
  source 1..10: note = CDR
QQSYNVPPFS

SEQ ID NO: 74 - protein, 11 aa, synthetic construct
  source 1..11: note = CDR
RASQGISTWLA

SEQ ID NO: 75 - protein, 10 aa, synthetic construct
  source 1..10: note = CDR
  VARIANT 5: note = X is N, Q, T or S; note (original language) = X选自N、Q、T或S
  VARIANT 6: note = X is T or V; note (original language) = X选自T或V
QQSYXXPPFS

SEQ ID NO: 76 - protein, 11 aa, synthetic construct
  source 1..11: note = CDR
  VARIANT 7: note = X is N, Q, T or S; note (original language) = X选自N、Q、T或S
  VARIANT 8: note = X is T or V; note (original language) = X选自T或V
RASQGIXXWLA

SEQ ID NO: 77 - protein, 446 aa, synthetic construct
  source 1..446: note = 2232-06 H1
QVQLVQSGAEVKKPGASVKVSCKASGYTFTSYGFSWVRQAPGQGLEWMGWISASNGNTYYAQKLQGRVTMTTDTSTSTAYMELRSLRSDDTAVYYCARVYADYADYWGQGTLVTVSSGGGGSSGAPRFLTRPKASVVSVGKDATLSCQIVGNPFPQVSWEKDKQPVTAGVRFRLAQDGDLYRLKILDLQLSDSGQYVCRARNAHGEAFACLGLQVDAEADKTHTCPPCPAPELLGGPSVFLFPPKPKDTLMISRTPEVTCVVVDVSHEDPEVKFNWYVDGVEVHNAKTKPREEQYNSTYRVVSVLTVLHQDWLNGKEYKCKVSNKALPAPIEKTISKAKGQPREPQVYTLPPCREEMTKNQVSLWCLVKGFYPSDIAVEWESNGQPENNYKTTPPVLDSDGSFFLYSKLTVDKSRWQQGNVFSCSVMHEALHNHYTQKSLSLSPGK

SEQ ID NO: 78 - protein, 210 aa, synthetic construct
  source 1..210: note = 2232-06 L1
DIQMTQSPSSVSASVGDRVTITCRASQGISTWLAWYQQKPGKAPKLLIYAASSLKSGVPSRFSGSGSGTDFTLTISSLQPEDFATYYCQQANSFPLTFGGGTKVEIKGGGGSGIPPKIECLPIDISIDEGKVLTVASAFTGEPTPEVTWSTGGRKIHSQEQGRFHIENTDDSTTLTIKDVQKQDGGLYTLTLRNEFGSDSATVNIHIRSI

SEQ ID NO: 79 - protein, 215 aa, synthetic construct
  source 1..215: note = 2232-06 L2
DIQMTQSPSSLSASIGDRATITCRASQHVGTYLNWYQQKPGKTPKLLISGAANLQSGVPSRFSGSGSGTDFTLTISSLQPEDFATYYCQQSYNVPPFSFGQGTKVEIKRTVAAPSVFIFPPSDEQLKSGTASVVCLLNNFYPREAKVQWKVDNALQSGNSQESVTEQDSKDSTYSLSSTLTLSKADYEKHKVYACEVTHQGLSSPVTKSFNRGEC

SEQ ID NO: 80 - protein, 447 aa, synthetic construct
  source 1..447: note = U3-1402 Ab H
QVQLQQWGAGLLKPSETLSLTCAVYGGSFSGYYWSWIRQPPGKGLEWIGEINHSGSTNYNPSLKSRVTISVETSKNQFSLKLSSVTAADTAVYYCARDKWTWYFDLWGRGTLVTVSSASTKGPSVFPLAPSSKSTSGGTAALGCLVKDYFPEPVTVSWNSGALTSGVHTFPAVLQSSGLYSLSSVVTVPSSSLGTQTYICNVNHKPSNTKVDKRVEPKSCDKTHTCPPCPAPELLGGPSVFLFPPKPKDTLMISRTPEVTCVVVDVSHEDPEVKFNWYVDGVEVHNAKTKPREEQYNSTYRVVSVLTVLHQDWLNGKEYKCKVSNKALPAPIEKTISKAKGQPREPQVYTLPPSREEMTKNQVSLTCLVKGFYPSDIAVEWESNGQPENNYKTTPPVLDSDGSFFLYSKLTVDKSRWQQGNVFSCSVMHEALHNHYTQKSLSLSPGK

SEQ ID NO: 81 - protein, 220 aa, synthetic construct
  source 1..220: note = U3-1402 Ab L
DIEMTQSPDSLAVSLGERATINCRSSQSVLYSSSNRNYLAWYQQNPGQPPKLLIYWASTRESGVPDRFSGSGSGTDFTLTISSLQAEDVAVYYCQQYYSTPRTFGQGTKVEIKRTVAAPSVFIFPPSDEQLKSGTASVVCLLNNFYPREAKVQWKVDNALQSGNSQESVTEQDSKDSTYSLSSTLTLSKADYEKHKVYACEVTHQGLSSPVTKSFNRGEC

SEQ ID NO: 82 - protein, 446 aa, synthetic construct
  source 1..446: note = S3 H
QVQLVESGGGVVQPGRSLRLSCAASGFSLSNYGVHWVRQAPGKGLEWLAVIWSGGSTNYAAAFVSRLTISKDNSKNTVYLQMNSLRAEDTAVYYCARNHDNPYNYAMDYWGQGTTVTVSSASTKGPSVFPLAPCSRSTSESTAALGCLVKDYFPEPVTVSWNSGALTSGVHTFPAVLQSSGLYSLSSVVTVPSSNFGTQTYTCNVDHKPSNTKVDKTVERKCCVECPPCPAPPVAGPSVFLFPPKPKDTLMISRTPEVTCVVVDVSHEDPEVQFNWYVDGVEVHNAKTKPREEQFNSTFRVVSVLTVVHQDWLNGKEYKCKVSNKGLPAPIEKTISKTKGQPREPQVYTLPPSREEMTKNQVSLTCLVKGFYPSDIAVEWESNGQPENNYKTTPPMLDSDGSFFLYSKLTVDKSRWQQGNVFSCSVMHEALHNHYTQKSLSLSPGK

SEQ ID NO: 83 - protein, 218 aa, synthetic construct
  source 1..218: note = S3 L
DIVLTQSPDSLAVSLGERATINCRADKSVSTSTYNYLHWYQQKPGQPPKLLIYLASNLASGVPDRFSGSGSGTDFTLTISSLQAEDVAVYYCQHSRDLPPTFGQGTKLEIKRTVAAPSVFIFPPSDEQLKSGTASVVCLLNNFYPREAKVQWKVDNALQSGNSQESVTEQDSKDSTYSLSSTLTLSKADYEKHKVYACEVTHQGLSSPVTKSFNRGEC

SEQ ID NO: 84 - protein, 447 aa, synthetic construct
  source 1..447: note = A13 H
QVQLVQSGAEVKKPGASVKVSCEASGYTFTSYGFSWVRQAPGQGLEWMGWISASNGNTYYAQKLQGRVTMTTDTSTSSAYMELRSLRSDDTAVYYCARVYADYADYWGQGTLVTVSSASTKGPSVFPLAPSSKSTSGGTAALGCLVKDYFPEPVTVSWNSGALTSGVHTFPAVLQSSGLYSLSSVVTVPSSSLGTQTYICNVNHKPSNTKVDKKVEPKSCDKTHTCPPCPAPELLGGPSVFLFPPKPKDTLMISRTPEVTCVVVDVSHEDPEVKFNWYVDGVEVHNAKTKPREEQYNSTYRVVSVLTVLHQDWLNGKEYKCKVSNKALPAPIEKTISKAKGQPREPQVYTLPPSREEMTKNQVSLTCLVKGFYPSDIAVEWESNGQPENNYKTTPPVLDSDGSFFLYSKLTVDKSRWQQGNVFSCSVMHEALHNHYTQKSLSLSPGK

SEQ ID NO: 85 - protein, 214 aa, synthetic construct
  source 1..214: note = A13 L
DIQMTQSPSSVSASVGDRVTITCRASQGINTWLAWYQQKPGKAPKLLIYAASSLKSGVPSRFSGSGSGADFTLTISSLQPEDFATYYCQQANSFPLTFGGGTKVEIKRTVAAPSVFIFPPSDEQLKSGTASVVCLLNNFYPREAKVQWKVDNALQSGNSQESVTEQDSKDSTYSLSSTLTLSKADYEKHKVYACEVTHQGLSSPVTKSFNRGEC

SEQ ID NO: 86 - protein, 447 aa, synthetic construct
  source 1..447: note = A H
QVQLVQSGGGLVQPGRSLRLSCAASGFTFDDYAMHWVRQAPGKGLEWVSGISWNSGSIGYADSVKGRFTISRDNAKNSLYLQMNSLRAEDTALYYCAKEGLPGLDYWGQGTLVTVSSASTKGPSVFPLAPSSKSTSGGTAALGCLVKDYFPEPVTVSWNSGALTSGVHTFPAVLQSSGLYSLSSVVTVPSSSLGTQTYICNVNHKPSNTKVDKKVEPKSCDKTHTCPPCPAPELLGGPSVFLFPPKPKDTLMISRTPEVTCVVVDVSHEDPEVKFNWYVDGVEVHNAKTKPREEQYNSTYRVVSVLTVLHQDWLNGKEYKCKVSNKALPAPIEKTISKAKGQPREPQVYTLPPSRDELTKNQVSLTCLVKGFYPSDIAVEWESNGQPENNYKTTPPVLDSDGSFFLYSKLTVDKSRWQQGNVFSCSVMHEALHNHYTQKSLSLSPGK

SEQ ID NO: 87 - protein, 215 aa, synthetic construct; identical to SEQ ID NO: 60
  source 1..215: note = A L

SEQ ID NO: 88 - protein, 5 aa, synthetic construct
  source 1..5: note = linker
GGNGT

SEQ ID NO: 89 - protein, 5 aa, synthetic construct
  source 1..5: note = linker
YGNGT

SEQ ID NO: 90 - protein, 5 aa, synthetic construct
  source 1..5: note = linker
EPKSS

SEQ ID NO: 91 - protein, 5 aa, synthetic construct
  source 1..5: note = linker
GGGGS

SEQ ID NO: 92 - protein, 10 aa, synthetic construct
  source 1..10: note = linker
GGGGSGGGGS

SEQ ID NO: 93 - protein, 15 aa, synthetic construct
  source 1..15: note = linker
GGGGSGGGGSGGGGS

SEQ ID NO: 94 - protein, 20 aa, synthetic construct
  source 1..20: note = linker
GGGGSGGGGSGGGGSGGGGS

SEQ ID NO: 95 - protein, 25 aa, synthetic construct
  source 1..25: note = linker
GGGGSGGGGSGGGGSGGGGSGGGGS

SEQ ID NO: 96 - protein, 98 aa, synthetic construct
  source 1..98: note = Titin-T
GIPPKIEALPSDISIDEGKVLTVACAFTGEPTPEVTWSCGGRKIHSQEQGRFHIENTDDLTTLIIMDVQKQDGGLYTLSLGNEFGSDSATVNIHIRSI

SEQ ID NO: 97 - protein, 97 aa, synthetic construct
  source 1..97: note = Obscurin-O
SGAPRFLTRPKAFVVSVGKDATLSCQIVGNPTPQVSWEKDQQPVAAGARFRLAQDGDLYRLTILDLALGDSGQYVCRARNAIGEAFAAVGLQVDAEA

SEQ ID NO: 98 - protein, 4 aa, synthetic construct
  source 1..4: note = linker
ASGS